European Patent Specification EP 3 407 704 B1, published August 14, 2024. Title: Reducing cadmium accumulation in field grown plants. Applicant: Philip Morris Products S.A. Application EP16153529.9. The sequence listing filed with the application follows.

SEQUENCE LISTING (64 sequences)

SEQ ID NO: 1 - protein, 1403 aa, Nicotiana tabacum
MVESEKMNETKKLSKSYFDVLGICCTSEVVLVEKILKNLEGVKEVSVIVTTKTVIVIHDSLLISPQQIVKALNQARLEASIRVKGEKNYQKKWPSPFAIGSGILLGLSFLKYFFAPFQWLALAAVAVGIPPIIFRGVAAVRNLTLDINILVLIAVAGSIVLHDYWEAGTIVFLFAIAEWLESRASHKATAAMSSLVNIVPPTAVLAESGEVVNVDEVKVNSILAVKAGETIPIDGVVVEGECDVDEKTLTGESFPVSKQRDSTVWAGTTNLNGYISVKTTALAEDCAVARMAQLVEDAQNKKSKTQRYIDKCAKYYTPAIVAISASLAIVPTALRVHNRNEWYRLALVTLVSACPCALVLSTPVAMCCALSKAATSGLLFKGAEYLETLAKIKIMAFDKTGTITKGEFMVTEFKSLIDGFSLNTLLYWVSSIESKSGHPMAAALVDYAQSNSVEPKPDRVEQFQNFPGEGIFGRIDGMEIYVGNRKISSRAGCTTVPEIEGDSFKGKSVGYIFLGSSPAGIFSLSDVCRIGVKEAMRELKQMGIKTAMLTGDCYAAANHVQDQLGGALDEFQAELLPEDKATIIKGFQKEAPTAMIGDGLNDAPALATADIGISMGISGSALAKETGHVILMTNDIGRIPKAARLARRVRRKIVENMIISVVTKAAIVALAIAGYPLVWAAVLADTGTCLLVILNSMLLLRGGTRRHGKKCWRSSTPSHAPHHKDKASCCKSENAPQLCCSDIESQKKCTSQSCSSEVCVPRCQPVSSGSKSCGNNQCPDSIENSGFHSHRRPQCCSSKMAAKACQSAVSESKSCGNNQCPDSVENSGFHSHPRPECCSSKMAAKACQSAVSESKSCGNNQCPDSVENSGFHSHPRPQCCSSKMAAKAGQSALSESKSCGNNNCSDSIHKSNCHSLTNSLVCSSKMSAPQCHSATSSNKSCGSTKCSDFSDKKCCQSDKIPQTCSTKKSAPGCQSAVSGSKSCGNSKCSDSKDNSSHPSHPDHQTCMSKLCAPQSQSATSSSRTCGNTKCSDTNSKNSCYSQTNSESCSSKMSGPSCKTANSGSRSCRNKKCQDSATENSFHSPLTNPLSGEKLSEQKSLDLVRKDKESSHDLRHGCSDEEHDHTNLDKAYDSCALQECCYSVQGNKTDVSETGIQETAHCDSTNQTCQTASSGSMTCGNDKILDSLSIHGCHSHDNPLHEENNLEQKILDVVGEGIKSPHAVGHGCSDKEHDHSHPEKAYDSCATDDCCFSVQVHGIDDVSKSEIQETAHCDSTKQSMVISSSCKHEPKDQVNHCGLHSKTTPTDEELAKLVRRCCKYKPCHDVRSGCRKHAAECGPTVRSTINILRDNHHHYLDCSGRKVCSLLEKRHIGGCCDSFRKECCAKKKHLGASFGGGLSEIVIE

SEQ ID NO: 2 - protein, 1444 aa, Nicotiana tabacum
MVESEKMNDTKNLSKSYFDVLGICCTSEVVLVEKILKNLEGVKEVSVIVTTKTVIVIHDSLLISQQQIVKALNQARLEASIRVKGEKNYQKKWPSPFAIGSGILLGLSFLKYFFAPFQWLALAAVAVGIPPIIFRGVAAVRNLTLDINILVLIAVTGSIVLHDYWEAGTIVFLFTIAEWLESRASHKATAAMSSLVNIVPPTAVLAESGEVVNVDEVKLNSILAVKAGETIPIDGVVMEGECDVDEKTLTGESFPVSKQIDSTVWAGTTNLNGYISVKTTALAEDCAVARMAQLVEDAQNKKSKTQRYIDKCAKYYTPAIVAISASLAIVPTALRVHNRNEWYRLALVTLVSACPCALVLSTPVAMCCALSKAATSGLLFKGAEYLETLAKIKIMAFDKTGTITRGEFMVTEFKSLVDGLGLNTLLYWVSSIESKSGHPMAAALVDYAQSNSVEPKPDRVEQFQNFPGEGIFGRIDGMEIYVGNRKISSRAGCTTVPEIEGDSFQGKSVGYIFLGSSPAGIFGLSDVCRIGVKEAMRELKQMGIKTAMLTGDCYAAANHVQDQLGGAMDEFQAELLPEDKATIIKGFQKEAPTAMIGDGLNDAPALATADIGISMGISGSALAKETGHVILMTNDIGRIPKAARLARRVRRKIVENMIISVVTKAAIVALAIAGYPLVWAAVLADTGTCLLVILNSMLLLRVGTHRHGKKCCRSATPSHAPNHKDKASCCKSENAPQLCCSDIESQKKCTSQSCSSEVCVPRCQPVSSGSKSCGNNQCPDSVENSGFHSHPRPQCCSSKMASKACQSAVSESKSCGNNQCPDSVENSGFHSHPRPQCCSSKMASKACQSAVSESKSCGNNQCPDSVENSGFHSHPRPQCCSLKMASKACQSAVSESKSCGNNQCPDSVENSGFHSHPRPQCCSSKMAAKACQSAVSESKSCGNNNCSESIYKSSCHSLTSSLVCSSKMSAPQCHSATSSSKSCGSTKCSNFSDKKCCQYDKIPQTCSTKKSAPGCQSAVSGSKSCGDSKCSDSKDNSSHPSHPDHQICTSKLCAPQSQSATSSSRTCGNMKCSDTNSKNSCYSHTNSESCSSKMSGPACKTANSGSRLCGNKKCLDSANENSFHSLTNPLCEEKLLEKESLDLARKDRESNHDLSHGCSDEEHDHLNLDKAHDSCALQECCYSVQGNKTDVSETGIQEAAHCDSINQTCQTAISGSMTCGNNKSLDSLSIHGCHSHDSPLHKESNLEQKSLDVAGEGIKSPHAVGQGCSDKEHNHSHPEKAYDSCATDDCCFSVQVHGIDDVSRSEIQETAHCDSTKQSTVIPSSCEHEPKDQVNHCGSHSKSIPTDEELAKLVRRCCKYKPCHDVRSGCRKHAAECGPTVRSTINILRDNHHHHLDCSGRKVCSLLEKRHIGGCCDSFRKECCAKNNHLGASFGGGLSEIVIE

SEQ ID NO: 3 - DNA, 4246 bp, Nicotiana tabacum
agagaaggagaaaaatggtggaaagtgaaaaaatgaatgaaacaaagaagttgagcaagagctattttgatgttttgggaatttgctgtacttcagaagttgttctagttgaaaaaattctcaagaatcttgaaggggttaaagaggtttcagtaattgtcacaacaaagactgtcattgttattcatgattctcttctcatttctccgcaacaaattgttaaagcattgaatcaagcaagattagaagcaagcataagagtgaaaggagagaaaaactaccaaaagaaatggccaagtccatttgcaattggcagtggaatattgcttggactctcatttttgaagtacttttttgcacctttccaatggttagcacttgcagctgttgcagttgggattcctccaattatttttagaggtgtggctgccgtgcgaaacctcactcttgacatcaacattcttgttttaatagcagtggctggatcaattgttttacacgattattgggaagctggtactattgtcttcttattcgccattgcagaatggctagagtcaagggcaagtcacaaggctaccgctgctatgtcatcactggtcaatatagtccctccaacagcagttttagctgaaagcggagaagtcgtaaatgttgatgaagtcaaggtgaatagcattcttgctgtgaaagctggtgaaactatacctattgatggagttgtagtggaaggggaatgtgacgtggacgagaaaacactgacaggcgagtcgtttccagtttctaagcaaagagattcaacggtctgggctggcactacaaatctaaatggctatatcagtgttaagactacggctttggctgaagattgtgcggtggctaggatggcacagcttgtcgaagatgctcagaacaagaaatcaaaaacccaaagatacatcgacaagtgtgctaaatattatacaccagcaattgtggctatatcagcttctttggcaattgttcctactgcattaagagttcacaatcgaaatgaatggtatcgcttggctttggtcacattggtgagtgcatgtccgtgtgcacttgttctatctacaccagttgccatgtgttgcgcactttcaaaagcagcaacgtccggtcttctgtttaaaggagcagagtaccttgagactctagctaaaatcaaaatcatggcttttgacaaaacagggactataactaaaggagaatttatggtgaccgagttcaagtctctgattgatggttttagtctcaatacactgctttactgggtttcaagcattgagagcaagtcaggtcatccgatggcagccgctctggtggactatgcacaatcaaattccgttgagccaaagcctgatagagttgagcagtttcaaaattttcctggtgaagggatatttggaagaattgatggaatggaaatctatgtcgggaataggaaaatttcttcaagagctggatgtaccacagtaccagaaatagagggtgatagtttcaaaggaaagtctgttggatacatatttttgggatcatctccagctggaattttcagtctttccgatgtttgtcgaattggtgtaaaagaagcaatgagagaactgaagcagatgggtatcaaaaccgcgatgcttactggtgattgttatgcagctgccaaccatgtgcaggatcagttaggtggagctttggatgaatttcaagcagaactcctaccagaggacaaggcaacaatcatcaagggttttcagaaggaagctccaacagcgatgataggcgacggccttaatgatgctcctgcattagcaacagctgacattggcatctcaatgggcatctctgggtcagctctcgctaaagaaacaggccatgttatactaatgacaaatgacatcggaagaataccgaaagctgcacgtcttgctagaagagttcgaaggaagattgttgagaatatgattatatcagtcgttacaaaggctgccatagttgcattggcaatagcaggttatccattggtttgggctgctgtcctcgcagatactgggacatgcttgctagtgattttgaacagcatgctacttctacgaggaggcacacgcagacatgggaaaaaatgttggagatcttctactccttcgcatgctccccaccacaaagacaaagcttcatgttgcaagtcggaaaatgctccccagctgtgttgctctgatattgagtcacaaaagaaatgtacaagtcaatcatgctcgtccgaggtgtgtgttccaagatgtcaacctgtctcctcaggatcaaagtcatgtggaaataatcagtgcccagactccattgaaaatagtggttttcattctcatcgccgtcctcaatgctgctcgtcgaagatggctgctaaagcatgccaatctgcagtttcagaatcaaagtcatgcggaaataatcagtgcccagactccgttgaaaatagtggttttcattctcatccccgtcctgaatgctgctcgtcgaagatggctgctaaagcgtgccaatctgcagtttcagaatcaaagtcatgtggaaataatcagtgcccagactccgttgaaaatagtggttttcattctcatccccgtcctcaatgctgttcatcgaagatggctgctaaagcaggccaatctgcactttcagaatcaaagtcatgtggaaataacaattgctcagactccattcacaagagtaattgtcattctttaactaactctctagtatgttcttccaagatgtctgctccacaatgtcattctgctacttcaagcaacaaatcatgtggaagtaccaagtgctccgacttcagtgacaaaaaatgttgtcaatccgacaaaattcctcaaacgtgctctaccaagaagtctgctccaggatgtcaatctgcagtttctgggtctaaatcatgtggaaatagcaagtgttcagactcaaaagacaatagtagccatccttcacatcccgatcatcaaacatgcatgtctaagttgtgtgctccacaaagccaatctgcaacttcaagctccaggacatgtggaaatacaaagtgctcggacaccaatagcaagaattcttgttattcacaaaccaactctgaatcatgctcttcaaagatgtctggtccatcatgcaaaactgctaattcaggttcaaggtcatgcagaaataagaagtgccaggactctgcaaccgagaacagttttcattcaccacttactaatccactcagtggggaaaagctttcggagcagaaaagcttggatttagtccgaaaagataaggaatcaagtcatgatcttcgtcatggctgctctgacgaggaacatgatcatacaaatttagacaaggcatatgacagttgtgccttacaagaatgttgttattcggttcaaggcaataaaactgatgtatcagaaactggaatccaggaaactgctcattgtgacagcaccaatcaaacatgccaaactgcaagttcaggatcgatgacatgcggaaatgataagatcctggactctctaagcatccatggttgtcattcgcatgataatccactccacgaggagaacaacttggagcagaaaatcttggatgttgttggagaaggtataaaatcacctcatgctgtcggtcatggctgttcggacaaggaacacgatcactcacatccagaaaaggcatatgacagttgtgcaacagatgattgttgtttttcagttcaagtccatggcattgacgacgtatcaaaaagtgaaattcaagaaactgctcattgtgacagcacaaagcagagcatggtcatctccagcagctgcaaacatgaaccaaaagatcaggtaaatcactgtggacttcactctaaaactactccaactgatgaagaactagccaagctggttagaagatgctgcaaatacaaaccatgccacgacgtccgttctggctgcaggaagcatgctgcagaatgtggtccaaccgttcgatcaaccatcaatatcttacgggacaaccatcatcattacctagactgcagtggtcgtaaggtttgttcgctgttggagaagagacacatcggtggatgctgtgacagcttcagaaaagaatgttgtgccaagaaaaaacaccttggagcaagttttggaggaggtttatcagaaattgtcatagagtagatgcaatccgaagtgtacat

SEQ ID NO: 4 - DNA, 4376 bp, Nicotiana tabacum
atagaaagaagagaatggtggaaagtgagaaaatgaatgacacaaagaatctgagcaagagctattttgatgttttgggaatttgctgtacttcagaagttgttcttgttgaaaaaattctcaagaatcttgaaggggttaaagaggtttcagtaattgtcacaacaaagactgtcattgttattcatgattctctcctcatttctcagcaacaaattgttaaagcattgaatcaagcaagattagaagcaagtataagagtgaaaggagagaaaaactaccaaaagaaatggccaagtccatttgcaattggcagtggaatattgcttggactctcatttttgaagtacttttttgcacctttccaatggttagcacttgcagctgttgcagttgggattcctccaattatttttaggggtgtggctgccgtgcgaaacctcactcttgacatcaacattcttgttttaatagcagtgacgggatcaattgttttacacgattattgggaagctggtactattgtcttcttattcaccattgcagaatggctagagtcaagggcaagtcacaaggctactgctgctatgtcatcactggtcaatatagtccctccaacagcagttttagctgaaagtggagaagtcgtaaatgttgatgaagtcaagttgaatagcattcttgctgttaaagctggtgaaactatacctattgatggagttgtaatggaaggggaatgtgacgtggacgagaaaacactgacaggcgagtcgtttccagtttctaagcaaatagattcaacggtctgggctggcactacaaatctaaatggctatatcagtgttaagactacggctttggctgaagattgtgcggtggctaggatggcgcagcttgtcgaagatgctcagaacaagaaatcaaaaacccaaagatacattgacaagtgtgctaaatattatacaccagcaattgtggctatatcagcttctttggcaatagttcctactgcattaagagttcacaatcgaaatgagtggtatcgcttggctttggtcacgttggtgagtgcatgtccgtgtgcacttgtgctatctacaccagttgccatgtgttgtgcactttctaaagcagcaacgtccggtcttctgtttaaaggagcagagtaccttgagactcttgctaaaatcaaaatcatggcttttgacaaaacagggactataactagaggagaatttatggtgaccgagttcaagtctctggttgatggtcttggtctcaatacactgctttactgggtttcaagtattgagagcaagtcaggtcatccgatggcagccgctctggttgactatgcacaatcaaattccgttgagccaaagcctgatagagttgagcagtttcaaaattttcctggtgaagggatatttggaagaattgatggaatggaaatctatgtcgggaataggaaaatttcttcaagagctggatgtactacagtaccagaaatagagggtgatagtttccaaggaaagtctgttggatacatatttttgggatcatctcccgctggaattttcggtctttccgatgtttgtcgaattggtgtaaaagaagcaatgagagagctgaagcagatgggtatcaaaaccgcgatgcttactggtgattgttatgcagctgccaaccatgtgcaggatcagttaggtggagctatggatgaatttcaagcggaactcttaccagaggacaaggcaacaatcatcaagggttttcagaaggaagctccaacagcgatgataggcgacggccttaatgatgctcctgcattagcaacagctgacattggcatctcaatgggcatctctgggtcagctctcgcgaaagaaacaggccatgttatactaatgacaaatgacatcggaagaataccaaaagctgcacgtcttgctagaagagttcgaaggaagattgttgagaatatgattatatcagtcgttacaaaggccgccatagttgcattggcaatagcaggttatccattggtttgggctgctgtcctcgcggatactgggacatgcttgctagtgatcttgaacagcatgctacttctacgagtaggcacacacagacatgggaaaaaatgttgtagatctgctactccttcgcatgctcccaaccacaaagacaaagcttcttgttgcaagtcggaaaatgctccgcagctgtgttgctctgatattgagtcacaaaagaaatgtacgagtcaatcatgctcgtccgaggtgtgtgttccaagatgtcaacctgtctcctcgggatcaaagtcatgtggaaataatcagtgcccagactccgttgaaaatagtggttttcattctcatccccgtcctcaatgctgctcgtcgaagatggcttctaaagcatgccaatctgcagtttcagaatcaaagtcatgtggaaataatcagtgcccagactccgttgaaaatagtggttttcattctcatccccgccctcaatgctgctcgtctaagatggcttctaaagcatgccaatctgcagtttcagaatcaaagtcatgtggaaataatcagtgcccagactccgttgaaaatagtggttttcattctcatccccgtcctcaatgctgctcgttgaagatggcttctaaagcatgccaatctgcagtttcagaatcaaagtcatgtggaaataatcagtgcccagactccgttgaaaatagtggttttcattctcatccccgtcctcaatgctgctcgtcgaagatggctgctaaagcatgccaatctgcagtttcagaatcaaagtcatgtggaaataacaattgctcggagtccatttacaagagtagttgtcattctttaacaagttctctagtatgttcttccaagatgtctgctccacaatgtcattctgccacttcaagctccaaatcatgtggaagtaccaagtgctccaacttcagtgacaaaaaatgttgccaatatgacaaaattcctcaaacgtgctctaccaagaagtctgctccaggatgtcaatctgcagtttctgggtctaaatcatgtggagatagcaagtgttcagactcgaaagacaatagtagccatccttcacatcccgatcatcaaatatgcacgtctaagttgtgtgctccacaaagccaatctgcaacttcaagctccaggacatgtggaaatatgaagtgctcggacaccaatagcaagaattcttgttattcacataccaactctgaatcatgctcttcaaagatgtctggtccagcatgcaaaactgctaattcaggttcaaggttatgcggaaataagaagtgcctagactctgcaaacgagaacagttttcattcacttactaatccactctgtgaggaaaagcttttggagaaggaaagcttggatttagcccgaaaagatagggaatcaaatcatgatcttagtcatggttgctctgacgaggaacatgatcatctaaatttagacaaggcacatgacagttgtgccttacaagaatgttgttattctgttcaaggcaataaaactgatgtatcagaaactggaatccaggaagctgctcattgtgacagcatcaatcaaacatgccaaactgcaatttcaggatcaatgacatgcggaaataataagagtctggactctctaagcatccatggttgtcattcacatgatagtccactccacaaggagagcaacttggagcagaaaagcttggatgttgctggagaaggtataaaatcacctcatgctgtcggtcaaggctgttcggacaaggagcacaatcactcgcatccagaaaaggcgtatgacagttgtgcaacagacgattgttgtttttcagttcaagtccatggcattgacgacgtatcaagaagtgaaattcaagaaactgctcattgtgacagcacaaaacagagcacggtcatccccagcagctgcgaacatgaaccaaaagatcaggtaaatcactgtggatctcactctaaaagtattccaactgatgaagaactagccaagctggttagaagatgctgcaaatacaaaccatgccacgatgtccgctctggctgcaggaagcatgctgcagaatgtggtccaaccgttcgatcaaccatcaatatcttacgggacaaccatcatcatcatctagactgcagtggtcgtaaggtttgttcgctgttggagaagagacacattggtggatgctgtgacagcttcagaaaagaatgttgtgccaagaacaatcaccttggagcaagttttggaggaggtttatcagaaattgtcatagagtagatgcaatctgaagtgtacatatgttgt

SEQ ID NO: 5 - DNA, 191 bp, Nicotiana tabacum
tgagagcaagtcaggtcatccgatggcagccgctctggtggactatgcacaatcaaattccgttgagccaaagcctgatagagttgagcagtttcaaaattttcctggtgaagggatatttggaagaattgatggaatggaaatctatgtcgggaataggaaaatttcttcaagagctggatgtaccacag

SEQ ID NO: 6 - DNA, 139 bp, Nicotiana tabacum
taaatggttgaatcatttcttatgctcatagtagagataaaacatcagagttataattataagtatatgatttctccagttaattttgctgttagattttctttgacctgtttagcactaatgcggtggatgtttgaat

SEQ ID NO: 7 - DNA, 23 bp, Artificial Sequence
  HMA4.1-Exon1 forward primer
gcatgttcttataagagaaactc

SEQ ID NO: 8 - DNA, 23 bp, Artificial Sequence
  HMA4.1-Exon1 reverse primer
gtgaatttatttaacaagccaca

SEQ ID NO: 9 - DNA, 22 bp, Artificial Sequence
  HMA4.1-Exon2 forward primer
ccaaaattgtttctgcttctcc

SEQ ID NO: 10 - DNA, 23 bp, Artificial Sequence
  HMA4.1-Exon2 reverse primer
cgtcatataaattgggacaaaag

SEQ ID NO: 11 - DNA, 23 bp, Artificial Sequence
  HMA4.1-Exon4/5 forward primer
gtgtctttattttctcactgata

SEQ ID NO: 12 - DNA, 23 bp, Artificial Sequence
  HMA4.1-Exon4/5 reverse primer
tagtgacgtgattcataagacaa

SEQ ID NO: 13 - DNA, 21 bp, Artificial Sequence
  HMA4.1-Exon6 forward primer
atcagtcctttcacttgaccc

SEQ ID NO: 14 - DNA, 22 bp, Artificial Sequence
  HMA4.1-Exon6 reverse primer
aaccattagagccatttcagaa

SEQ ID NO: 15 - DNA, 23 bp, Artificial Sequence
  HMA4.1-Exon7/8 forward primer
gatactgcaatacaaaagcacat

SEQ ID NO: 16 - DNA, 22 bp, Artificial Sequence
  HMA4.1-Exon7/8 reverse primer
cacttacttggtaatacgttct

SEQ ID NO: 17 - DNA, 20 bp, Artificial Sequence
  HMA4.2-Exon1 forward primer
ttgctactctgggttgctac

SEQ ID NO: 18 - DNA, 23 bp, Artificial Sequence
  HMA4.2-Exon1 reverse primer
tcaagtttaaagtttgcttctac

SEQ ID NO: 19 - DNA, 22 bp, Artificial Sequence
  HMA4.2-Exon2 forward primer
tgtgcatacataacgtaaatcg

SEQ ID NO: 20 - DNA, 22 bp, Artificial Sequence
  HMA4.2-Exon2 reverse primer
atcaaataccacataagtaggg

SEQ ID NO: 21 - DNA, 23 bp, Artificial Sequence
  HMA4.2-Exon4/5 forward primer
tttagtcactttgacataaatgg

SEQ ID NO: 22 - DNA, 22 bp, Artificial Sequence
  HMA4.2-Exon4/5 reverse primer
aagacagagaacaagttcacat

SEQ ID NO: 23 - DNA, 20 bp, Artificial Sequence
  HMA4.2-Exon6 forward primer
tcagtcctttcgcttgacct

SEQ ID NO: 24 - DNA, 20 bp, Artificial Sequence
  HMA4.2-Exon6 reverse primer
gagaatgtggtactcgcaag

SEQ ID NO: 25 - DNA, 22 bp, Artificial Sequence
  HMA4.2-Exon7/8 forward primer
atacattgaggacacataatcg

SEQ ID NO: 26 - DNA, 21 bp, Artificial Sequence
  HMA4.2-Exon7/8 reverse primer
tataccccattctgacccttg

SEQ ID NO: 27 - DNA, 24 bp, Artificial Sequence
  HMA4.1 forward primer
tcatgcagaaataagaagtgccag

SEQ ID NO: 28 - DNA, 23 bp, Artificial Sequence
  HMA4.1 reverse primer
atggatgcttagagagtccagga

SEQ ID NO: 29 - DNA, 25 bp, Artificial Sequence
  HMA4.2 forward primer
gttatgcggaaataagaagtgccta

SEQ ID NO: 30 - DNA, 24 bp, Artificial Sequence
  HMA4.2 reverse primer
catggatgcttagagagtccagac

SEQ ID NO: 31 - DNA, 24 bp, Artificial Sequence
  Actin 9 forward primer
ctattctccgctttggacttggca

SEQ ID NO: 32 - DNA, 23 bp, Artificial Sequence
  Actin 9 reverse primer
aggacctcaggacaacggaaacg

SEQ ID NO: 33 - DNA, 14 bp, Artificial Sequence
  HMA4.1 Q293* mutant-probe
aggatggcacagct

SEQ ID NO: 34 - DNA, 14 bp, Artificial Sequence
  HMA4.1 wild type probe
aggatggcacagct

SEQ ID NO: 35 - DNA, 35 bp, Artificial Sequence
  HMA4.1 forward primer
ctggcactacaaatctaaatggtagtatagtattt

SEQ ID NO: 36 - DNA, 29 bp, Artificial Sequence
  HMA4.1 reverse primer
ctggtgtataatatttagcacacttgtcg

SEQ ID NO: 37 - DNA, 15 bp, Artificial Sequence
  HMA4.1 E296K mutant-probe
cacagcttgtcaaag

SEQ ID NO: 38 - DNA, 15 bp, Artificial Sequence
  HMA4.1 wild type probe
cacagcttgtcgaag

SEQ ID NO: 39 - DNA, 35 bp, Artificial Sequence; identical to SEQ ID NO: 35
  HMA4.1 forward primer

SEQ ID NO: 40 - DNA, 29 bp, Artificial Sequence
  HMA4.1 reverse primer
ctggtgtataatatttagcacacttgtcg

SEQ ID NO: 41 - DNA, 19 bp, Artificial Sequence
  HMA4.1 T402I mutant-probe
tttgacaaaacagggatta

SEQ ID NO: 42 - DNA, 19 bp, Artificial Sequence
  HMA4.1 wild type probe
tttgacaaaacagggacta

SEQ ID NO: 43 - DNA, 20 bp, Artificial Sequence
  HMA4.1 forward primer
ccatgtgttgcgcactttca

SEQ ID NO: 44 - DNA, 25 bp, Artificial Sequence
  HMA4.1 reverse primer
aactcggtcaccataaattctcctt

SEQ ID NO: 45 - DNA, 18 bp, Artificial Sequence
  HMA4.1 G251D mutant-probe
agaaaacactgacagacg

SEQ ID NO: 46 - DNA, 16 bp, Artificial Sequence
  HMA 4.1 wild type probe
aaaacactgacaggcg

SEQ ID NO: 47 - DNA, 27 bp, Artificial Sequence
  HMA 4.1 forward primer
aagtcgtaaatgttgatgaagtcaagg

SEQ ID NO: 48 - DNA, 21 bp, Artificial Sequence
  HMA 4.1 reverse primer
cagcccagaccgttgaatctc

SEQ ID NO: 49 - DNA, 18 bp, Artificial Sequence
  HMA4.1 V351M mutant-probe
ctttggtcacattgatga

SEQ ID NO: 50 - DNA, 18 bp, Artificial Sequence
  HMA 4.1 wild type probe
ttggtcacattggtgagt

SEQ ID NO: 51 - DNA, 25 bp, Artificial Sequence
  HMA 4.1 forward primer
ggctatatcagcttctttggcaatt

SEQ ID NO: 52 - DNA, 26 bp, Artificial Sequence
  HMA 4.1 reverse primer
aacacatggcaactggtgtagataga

SEQ ID NO: 53 - DNA, 20 bp, Artificial Sequence
  HMA4.1 G382R mutant-probe
ttctgtttaaaagagcagag

SEQ ID NO: 54 - DNA, 21 bp, Artificial Sequence
  HMA 4.1 wild type probe
tctgtttaaaggagcagagta

SEQ ID NO: 55 - DNA, 20 bp, Artificial Sequence
  HMA 4.1 forward primer
ccatgtgttgcgcactttca

SEQ ID NO: 56 - DNA, 25 bp, Artificial Sequence
  HMA 4.1 reverse primer
aactcggtcaccataaattctcctt

SEQ ID NO: 57 - DNA, 19 bp, Artificial Sequence
  HMA4.2 W265* mutant-probe
atagattcaacggtctagg

SEQ ID NO: 58 - DNA, 15 bp, Artificial Sequence
  HMA 4.2 wild type probe
ttcaacggtctgggc

SEQ ID NO: 59 - DNA, 31 bp, Artificial Sequence
  HMA 4.2 forward primer
ggtgaaactatacctattgatggagttgtaa

SEQ ID NO: 60 - DNA, 32 bp, Artificial Sequence
  HMA 4.2 reverse primer
cactaaataaatgaagcatgaaggaatactac

SEQ ID NO: 61 - DNA, 16 bp, Artificial Sequence
  HMA4.2 Q561* mutant-probe
caaccatgtgtaggat

SEQ ID NO: 62 - DNA, 16 bp, Artificial Sequence
  HMA 4.2 wild type probe
tgccaaccatgtgcag

SEQ ID NO: 63 - DNA, 26 bp, Artificial Sequence
  HMA 4.2 forward primer
ttggtgtaaaagaagcaatgagagag

SEQ ID NO: 64 - DNA, 25 bp, Artificial Sequence
  HMA 4.2 reverse primer
atcatttcagcgtattgcagaattt